European Patent Application EP 4 488 376 A1, published January 8, 2025. Title: Verfahren zur Herstellung einer wässerigen Lösung enthaltend L-Sorbose. Applicant: Annikki GmbH. The sequence listing filed with the application follows.

SEQUENCE LISTING (6 sequences)

SEQ ID NO: 1 - protein, 320 aa, Rasamsonia emersonii
MATPTIKLNSGYDMPLVGFGLWKVNRETCADQVYEAIKAGYRLFDGACDYGNEVEAGQGVARAIKEGIVKREDLFIVSKLWNTFHEADKVEPIARKQLADWGLDYFDLYLIHFPIALKYVDPAEIYPPGWTGTKKEVEFSNATIQETWQAMETLVDKKLTRSIGISNFSAQLIMDLLRYARIRPATLQIEHHPYLTQQALVEYVQKEGIAVTAYSSFGPLSFLELGHQVAKDTPLLFEHSTVKSIAEKHGKTPAQVLLRWATQRNIAVIPKSNNPGRLAQNLDVTAWDLEPADIEALSALNKNLRFNNPPSYGLYIPIFA

SEQ ID NO: 2 - DNA, 963 bp, Rasamsonia emersonii
  source 1..963: mol_type = genomic DNA
atggccacgcctactatcaagctgaacagcggctatgacatgcccctggtgggctttggtctgtggaaggtcaacagggaaacctgcgcggaccaggtctacgaggctatcaaggcgggctaccgcttgtttgacggtgcgtgcgactatggcaacgaagttgaggccggccagggtgtcgctcgcgccatcaaggaaggcattgtgaagcgtgaggacctcttcattgtgtccaagctgtggaacacgttccacgaggccgacaaggtcgagccgatcgcgcggaagcagctggccgactggggcctcgactactttgacctgtacctcatccacttcccgatcgcgctgaagtacgtcgacccggccgagatctacccgccgggctggacgggcaccaagaaggaggtcgagttcagcaacgcgacgatccaggagacgtggcaggccatggagaccctggtcgacaagaagctgacgcgcagcatcggcatcagcaacttcagcgcccagctgatcatggacctgctgcggtacgcgcgcatccgccccgcgaccttgcagatcgagcaccacccgtacctgacgcagcaggcgctggtcgagtacgtgcagaaggagggcatcgccgtgacggcgtactcgtccttcggcccactgagcttcctggaactgggccaccaggtcgccaaggacacgccgctgctcttcgagcactcgaccgtcaagtcgatcgccgagaagcacggcaagacgcccgcccaggtgctactgcgctgggccacccagcgcaacatcgccgtcatccccaagagcaacaacccgggccgcctggcgcagaacctggacgtgacggcgtgggatctggagcccgccgacattgaggccttgagcgcgctgaacaagaaccttcgattcaacaacccacctagctacggactgtacatcccgatcttcgcttaa

SEQ ID NO: 3 - protein, 325 aa, Thermochaetoides thermophila
MAPQIPNIKLSSGYDMPQVGFGLWKVDRSICADVVYNAIKIGYRLFDGACDYGNEVEAGQGIARAIKEGIVKREELFIVSKLWNTFHDGDKVEPIVRKQLADWGIDYFDLYLVHFPVALEYVDPSVRYPPGWFYDGEKEIRPSKATIQETWTAMESLVEKGLARSIGVSNFQAQLLYDLLRYAKIRPATLQIEHHPFLVQQELLNLAKAEGIAVTAYSSFGPQSFLEFNMKHAVQLTPLFEDETIKKIAAKYNRPASQVLLRWATQRGLAIIPKSTRPEIMKSNLESIEFDLSEEDIATISAFDRGLRFNQPTNYFPTEHLWIFG

SEQ ID NO: 4 - DNA, 978 bp, Thermochaetoides thermophila
  source 1..978: mol_type = genomic DNA
atggctccccagatccccaacattaagctcagcagcggctatgacatgccccaggtgggctttggactgtggaaggtcgaccgctcgatctgcgccgacgtcgtctacaacgcaattaagattggctaccgcctgtttgacggcgcttgcgactatggcaacgaagtcgaggccggccagggcattgcccgcgccatcaaggagggcatcgtgaagcgtgaggagctcttcatcgtgtccaagctctggaacaccttccacgacggcgacaaggtcgagcccatcgtccgcaagcagctcgccgactggggcattgactacttcgacctctacctcgtccacttccctgtcgccctcgagtacgtcgacccctcggtccgctacccgcccggctggttctacgatggcgagaaggagatccgccccagcaaggccaccatccaggagacctggaccgccatggagtcgctcgttgagaagggtctggcccgcagcattggtgtctccaacttccaggcccagctcctctacgacctgctgcgctacgccaagatccgcccggccacccttcagatcgagcatcaccccttcctcgtccagcaggagctgctcaacctggccaaggccgagggcattgccgtgactgcctacagctcattcggccctcagagcttcctcgagttcaacatgaagcacgccgtgcagctcaccccgctcttcgaggacgagaccatcaagaagatcgccgccaagtacaaccgtcctgcttcgcaggttctcctgcgctgggccactcagcgcggtctggccattatccccaagagcacgcgccccgagatcatgaagtccaacctcgagagcatcgagttcgacctcagcgaggaagatattgccaccatctcggccttcgaccgcggcctgcgcttcaaccagcccacaaactacttccccaccgagcacctctggatctttggctaa

SEQ ID NO: 5 - protein, 494 aa, Sinorhizobium meliloti
MATKFSLATLDAVKATAGVPNYGRHDLRAGIVHFGVGNFHRAHQAVYLDDLFNLGRDRDWAIIGAGVLPSDKVMRDKLEAQDFLTTVVEQDNNRTGAHVTGAMIAYLEPGDTPAIVAQLASPLIRIVSLTITEGGYFIDPASGVFDPAHPAIVEDARDPAAPKTVFGLILAGLAERRAKGIPPFTIMSCDNIPGNGEVTHAAVSGLARLSDPGFADWIDANVAFPNGMVDRITPATGAREIGIVASQYGIDDAWPVFCEEFKQWVLEDRFPQGRPALEEVGVQFVPDVAPYEHMKIRILNGGHAAIAYPAALLDIHFVHEAMEEPLIRAFLSKLEHDEIIPVIPPVPDTDLKDYYKLIETRFSNPKIGDTVARLAQDGSNRQPKFILPSTADRLRRGEDVVGLSLVSALWCRYFAGKSDSGKEIVFNDANADRLHAAAVAAKDDPMAFLALSDIFGDVAQSDLFRRRFAHALKVLWEKGTRATLQLYLDGNLGE

SEQ ID NO: 6 - DNA, 1485 bp, Sinorhizobium meliloti
  source 1..1485: mol_type = genomic DNA
atggcgaccaaattctcccttgccacgctcgacgcggtcaaagccacggccggcgtcccgaactacggccggcatgaccttcgggccggcatcgtgcacttcggcgtcggcaatttccaccgcgcgcatcaggcggtctatctcgatgaccttttcaacctgggacgcgatcgcgattgggcgatcatcggcgcgggtgtcctgccatcggacaaggtcatgcgcgacaagctcgaagcgcaggatttcctgacgacggtggtcgagcaggacaacaaccgcacgggcgcgcatgtcaccggcgccatgatcgcctacctcgagcccggcgacacgcccgcgatcgtggcgcagctcgcgagcccgctcatccgcatcgtctccctgacgatcaccgaaggcggctatttcatcgatccggcatccggcgtcttcgacccggcgcatccggcgatcgtcgaggatgcgcgcgatccggcggctccaaaaaccgtcttcggcctcatcctggcagggctcgccgaacgccgcgccaagggtattccgccgttcacgatcatgtcctgcgacaatattcctggaaacggggaggtcacccacgctgccgtttccggtctggcgcgcctttccgatccaggctttgcggactggatcgatgccaatgtcgcctttccgaacggcatggtcgatcgcatcacgccggcgaccggtgcccgcgagatcggcatcgtcgcctcgcaatacggaatcgacgatgcctggccggtcttttgcgaggaattcaagcaatgggtgctggaagaccgcttcccgcaaggccgcccggcgctggaagaggtgggcgttcagttcgtgcccgacgtggcgccgtacgagcacatgaagatccgtatcctcaacggcggccatgcggcgatcgcctatccggcggcactgctcgacatccatttcgttcatgaggcgatggaggagccgttgatccgcgccttcctgtcaaagctggagcacgacgagatcatcccggtgataccgcccgttccggacacggatctgaaggattattacaagctcatcgagacgcgtttctccaatccgaagatcggcgacacggtcgcgcggctggcgcaggacggctccaaccgacagccgaaattcatcctgccgtcgacggccgaccgcctgcgccgcggcgaagacgtcgtcgggttgtcgctcgtttcggcgctgtggtgccgctatttcgccggcaagtcggacagcggcaaggagatcgttttcaacgacgccaacgccgaccggctgcatgccgccgcggttgcagcgaaggacgatccaatggcgttccttgcgctttccgacatcttcggcgatgtcgcgcaatccgatctcttccgccgccgtttcgctcacgcgttgaaagtgctttgggaaaagggtacgcgtgccacgctccagctttatctggacggaaacctcggggaataa